European Patent Application EP 4 261 223 A1, published October 18, 2023. Title: ANTI-SIRPα ANTIBODY AND APPLICATION THEREOF. Applicant: BioRay Pharmaceutical Co., Ltd. Hisun Biopharmaceutical Co., Ltd. The sequence listing filed with the application follows.

SEQUENCE LISTING (42 sequences)

SEQ ID NO: 1 - protein, 113 aa, Artificial Sequence
  #4 VH
EVQLVQSGAEVKKPGATVKISCRGSGFNIKDYYIQWVQQAPGKGLEWMGWIDPENGDTKYAPKFQGRVTITADTSTDTAYMELSSLRSEDTAVYYCYAKGPYWGQGTTLTVSS

SEQ ID NO: 2 - DNA, 339 bp, Artificial Sequence
  #4 VH DNA
gaggtgcagctggtgcagtccggcgccgaggtgaagaagcccggcgccaccgtgaagatctcctgccgcggctccggcttcaacatcaaggactactacatccagtgggtgcagcaggcccccggcaagggcctggagtggatgggctggatcgaccccgagaacggcgacaccaagtacgcccccaagttccagggccgcgtgaccatcaccgccgacacctccaccgacaccgcctacatggagctgtcctccctgcgctccgaggacaccgccgtgtactactgctacgccaagggcccctactggggccagggcaccaccctgaccgtctcgagc

SEQ ID NO: 3 - protein, 5 aa, Artificial Sequence
  #4 VH-CDR1
DYYIQ

SEQ ID NO: 4 - protein, 17 aa, Artificial Sequence
  #4 VH-CDR2
WIDPENGDTKYAPKFQG

SEQ ID NO: 5 - protein, 4 aa, Artificial Sequence
  #4 VH-CDR3
KGPY

SEQ ID NO: 6 - protein, 113 aa, Artificial Sequence
  #4 VL
DIVMTQSPDSLAVSLGERATINCKSSQSLFYSSNQKNFLAWYQQKPGQPPKLLIYWASTRESGVPDRFTGSGSGTDFTLTISSVKAEDLAVYYCQQYYSYPPTFGGGTKLEIK

SEQ ID NO: 7 - DNA, 339 bp, Artificial Sequence
  #4 VL DNA
gacatcgtgatgacccagtcccccgactccctggccgtgtccctgggcgagcgcgccaccatcaactgcaagtcctcccagtccctgttctactcctccaaccagaagaacttcctggcctggtaccagcagaagcccggccagccccccaagctgctgatctactgggcctccacccgcgagtccggcgtgcccgaccgcttcaccggctccggctccggcaccgacttcaccctgaccatctcctccgtgaaggccgaggacctggccgtgtactactgccagcagtactactcctacccccccaccttcggcggcggcaccaagctcgagataaaa

SEQ ID NO: 8 - protein, 17 aa, Artificial Sequence
  #4 VL-CDR1
KSSQSLFYSSNQKNFLA

SEQ ID NO: 9 - protein, 7 aa, Artificial Sequence
  #4 VL-CDR2
WASTRES

SEQ ID NO: 10 - protein, 9 aa, Artificial Sequence
  #4 VL-CDR3
QQYYSYPPT

SEQ ID NO: 11 - protein, 118 aa, Artificial Sequence
  #11 VH
QVTLKESGPVLVKPTETLTLTCTVSGFSLSSHGVHWIRQPPGKALEWLAVIWSDGSTTYNSTLKSRLTISKDTSKSQVVLTMTNMDPVDTATYYCARHGNYHYNMDYWGQGTLVTVSS

SEQ ID NO: 12 - DNA, 354 bp, Artificial Sequence
  #11 VH DNA
caggtgaccctgaaggagtccggccccgtgctggtgaagcccaccgagaccctgaccctgacctgcaccgtgtccggcttctccctgtcctcccacggcgtgcactggatccgccagccccccggcaaggccctggagtggctggccgtgatctggtccgacggctccaccacctacaactccaccctgaagtcccgcctgaccatctccaaggacacctccaagtcccaggtggtgctgaccatgaccaacatggaccccgtggacaccgccacctactactgcgcccgccacggcaactaccactacaacatggactactggggccagggcaccctggtgaccgtctcgagc

SEQ ID NO: 13 - protein, 5 aa, Artificial Sequence
  #11 VH-CDR1
SHGVH

SEQ ID NO: 14 - protein, 16 aa, Artificial Sequence
  #11 VH-CDR2
VIWSDGSTTYNSTLKS

SEQ ID NO: 15 - protein, 10 aa, Artificial Sequence
  #11 VH-CDR3
HGNYHYNMDY

SEQ ID NO: 16 - protein, 108 aa, Artificial Sequence
  #11 VL
DIQLTQSPSFLSASVGDRVTITCRTSSRVNSGYLHWYQQKPGKAPKLLIYSTSTLASGVPSRFSGSGSGTEFTLTISSLQPEDFATYYCQQYSSYPWTFGGGTKLEIK

SEQ ID NO: 17 - DNA, 324 bp, Artificial Sequence
  #11 VL DNA
gacatccagctgacccagtccccctccttcctgtccgcctccgtgggcgaccgcgtgaccatcacctgccgcacctcctcccgcgtgaactccggctacctgcactggtaccagcagaagcccggcaaggcccccaagctgctgatctactccacctccaccctggcctccggcgtgccctcccgcttctccggctccggctccggcaccgagttcaccctgaccatctcctccctgcagcccgaggacttcgccacctactactgccagcagtactcctcctacccctggaccttcggcggcggcaccaagctcgagataaaa

SEQ ID NO: 18 - protein, 12 aa, Artificial Sequence
  #11 VL-CDR1
RTSSRVNSGYLH

SEQ ID NO: 19 - protein, 7 aa, Artificial Sequence
  #11 VL-CDR2
STSTLAS

SEQ ID NO: 20 - protein, 9 aa, Artificial Sequence
  #11 VL-CDR3
QQYSSYPWT

SEQ ID NO: 21 - protein, 122 aa, Artificial Sequence
  #13 VH
QVQLVQSGSELKKPGASVKVSCKASGYTFTDYSIHWVRQAPGQGLEWMGWINTETGEPTYADDFKGRFVFSLDTSVSTAYLQICSLKAEDTAVYYCSRGPLYRYDGYGLEYWGQGTLVTVSS

SEQ ID NO: 22 - DNA, 366 bp, Artificial Sequence
  #13 VH DNA
caggtgcagctggtgcagtccggctccgagctgaagaagcccggcgcctccgtgaaggtgtcctgcaaggcctccggctacaccttcaccgactactccatccactgggtgcgccaggcccccggccagggcctggagtggatgggctggatcaacaccgagaccggcgagcccacctacgccgacgacttcaagggccgcttcgtgttctccctggacacctccgtgtccaccgcctacctgcagatctgctccctgaaggccgaggacaccgccgtgtactactgctcccgcggccccctgtaccgctacgacggctacggcctggagtactggggccagggcaccctggtgaccgtctcgagc

SEQ ID NO: 23 - protein, 5 aa, Artificial Sequence
  #13 VH-CDR1
DYSIH

SEQ ID NO: 24 - protein, 17 aa, Artificial Sequence
  #13 VH-CDR2
WINTETGEPTYADDFKG

SEQ ID NO: 25 - protein, 13 aa, Artificial Sequence
  #13 VH-CDR3
GPLYRYDGYGLEY

SEQ ID NO: 26 - protein, 107 aa, Artificial Sequence
  #13 VL
DIVMTQSPDSLAVSLGERATINCKASQSVSNDVAWYQQKPGQPPKLLIYYASNRCTGVPDRFSGSGSGTDFTLTISSLQAEDVAVYYCHQDYISPYTFGGGTKLEIK

SEQ ID NO: 27 - DNA, 321 bp, Artificial Sequence
  #13 VL DNA
gacatcgtgatgacccagtcccccgactccctggccgtgtccctgggcgagcgcgccaccatcaactgcaaggcctcccagtccgtgtccaacgacgtggcctggtaccagcagaagcccggccagccccccaagctgctgatctactacgcctccaaccgctgcaccggcgtgcccgaccgcttctccggctccggctccggcaccgacttcaccctgaccatctcctccctgcaggccgaggacgtggccgtgtactactgccaccaggactacatctccccctacaccttcggcggcggcaccaagctcgagataaaa

SEQ ID NO: 28 - protein, 11 aa, Artificial Sequence
  #13 VL-CDR1
KASQSVSNDVA

SEQ ID NO: 29 - protein, 7 aa, Artificial Sequence
  #13 VL-CDR2
YASNRCT

SEQ ID NO: 30 - protein, 9 aa, Artificial Sequence
  #13 VL-CDR3
HQDYISPYT

SEQ ID NO: 31 - protein, 118 aa, Artificial Sequence
  #14 VH
QVQLQESGPGLVKPSQTLSLTCTVSGGSISSGYYWSWIRQHPGKGLEWIGYISYDGSRYNNPSLKNRVTISVDTSKNQFSLKLSSVTAADTAVYYCAREEYANYFAYWGQGTTVTVSS

SEQ ID NO: 32 - DNA, 354 bp, Artificial Sequence
  #14 VH DNA
caggtgcagctgcaggagagcggaccaggactggtgaagcctagccagacactgtctctgacctgcacagtgagcggcggctctatctccagcggctactattggtcttggatcagacagcacccaggcaagggcctggagtggatcggctacatctcctatgatggcagcaggtataacaatccttccctgaagaaccgggtgaccatctctgtggacacatccaagaatcagttcagcctgaagctgtcttccgtgaccgccgctgatacagccgtgtactattgcgctcgcgaggagtacgccaactatttcgcttactggggccagggcaccacagtgaccgtgagctct

SEQ ID NO: 33 - protein, 6 aa, Artificial Sequence
  #14 VH-CDR1
SGYYWS

SEQ ID NO: 34 - protein, 16 aa, Artificial Sequence
  #14 VH-CDR2
YISYDGSRYNNPSLKN

SEQ ID NO: 35 - protein, 9 aa, Artificial Sequence
  #14 VH-CDR3
EEYANYFAY

SEQ ID NO: 36 - protein, 113 aa, Artificial Sequence
  #14 VL
DIVMTQSPDSLAVSLGERATINCKSSQSLFYSSNQKNFLAWYQQKPGQPPKLLIYWASTRESGVPDRFTGSGSGTDFTLTISSVKAEDLAVYYCQQYYSYPPTFGQGTKLEIK

SEQ ID NO: 37 - DNA, 339 bp, Artificial Sequence
  #14 VL DNA
gatatcgtgatgacccagtctcctgactccctggccgtgagcctgggcgagagagctacaatcaactgtaagtccagccagtctctgttctactcttccaaccagaagaattttctggcctggtatcagcagaagcccggccagccccctaagctgctgatctactgggctagcaccagagagtctggagtgcctgaccgcttcaccggatccggaagcggaacagacttcaccctgacaatcagctctgtgaaggccgaggatctggccgtgtactattgccagcagtactattcttatccacccaccttcggccagggcacaaagctcgagatcaag

SEQ ID NO: 38 - protein, 17 aa, Artificial Sequence
  #14 VL-CDR1
KSSQSLFYSSNQKNFLA

SEQ ID NO: 39 - protein, 7 aa, Artificial Sequence
  #14 VL-CDR2
WASTRES

SEQ ID NO: 40 - protein, 9 aa, Artificial Sequence
  #14 VL-CDR3
QQYYSYPPT

SEQ ID NO: 41 - protein, 448 aa, Artificial Sequence
  #14 HC
QVQLQESGPGLVKPSQTLSLTCTVSGGSISSGYYWSWIRQHPGKGLEWIGYISYDGSRYNNPSLKNRVTISVDTSKNQFSLKLSSVTAADTAVYYCAREEYANYFAYWGQGTTVTVSSASTKGPSVFPLAPSSKSTSGGTAALGCLVKDYFPEPVTVSWNSGALTSGVHTFPAVLQSSGLYSLSSVVTVPSSSLGTQTYICNVNHKPSNTKVDKKVEPKSCDKTHTCPPCPAPELLGGPSVFLFPPKPKDTLMISRTPEVTCVVVDVSHEDPEVKFNWYVDGVEVHNAKTKPREEQYASTYRVVSVLTVLHQDWLNGKEYKCKVSNKALPAPIEKTISKAKGQPREPQVYTLPPSREEMTKNQVSLTCLVKGFYPSDIAVEWESNGQPENNYKTTPPVLDSDGSFFLYSKLTVDKSRWQQGNVFSCSVMHEALHNHYTQKSLSLSPGK

SEQ ID NO: 42 - protein, 220 aa, Artificial Sequence
  #14 LC
DIVMTQSPDSLAVSLGERATINCKSSQSLFYSSNQKNFLAWYQQKPGQPPKLLIYWASTRESGVPDRFTGSGSGTDFTLTISSVKAEDLAVYYCQQYYSYPPTFGQGTKLEIKRTVAAPSVFIFPPSDEQLKSGTASVVCLLNNFYPREAKVQWKVDNALQSGNSQESVTEQDSKDSTYSLSSTLTLSKADYEKHKVYACEVTHQGLSSPVTKSFNRGEC